European Patent Application EP 4 194 472 A1, published June 14, 2023. Title: 包含新型共刺激结构域的嵌合抗原受体及其用途. Applicant: 南京北恒生物科技有限公司. The sequence listing filed with the application follows.

SEQUENCE LISTING (44 sequences)

SEQ ID NO: 1 - protein, 242 aa, Artificial Sequence
  CD19 scFv-1
DIQMTQTTSSLSASLGDRVTISCRASQDISKYLNWYQQKPDGTVKLLIYHTSRLHSGVPSRFSGSGSGTDYSLTISNLEQEDIATYFCQQGNTLPYTFGGGTKLEITGGGGSGGGGSGGGGSEVKLQESGPGLVAPSQSLSVTCTVSGVSLPDYGVSWIRQPPRKGLEWLGVIWGSETTYYNSALKSRLTIIKDNSKSQVFLKMNSLQTDDTAIYYCAKHYYYGGSYAMDYWGQGTSVTVSS

SEQ ID NO: 2 - DNA, 726 bp, Artificial Sequence
  CD19 scFv-1
gacatccagatgacacagactacatcctccctgtctgcctctctgggagacagagtcaccatcagttgcagggcaagtcaggacattagtaaatatttaaattggtatcagcagaaaccagatggaactgttaaactcctgatctaccatacatcaagattacactcaggagtcccatcaaggttcagtggcagtgggtctggaacagattattctctcaccattagcaacctggagcaagaagatattgccacttacttttgccaacagggtaatacgcttccgtacacgttcggaggggggaccaagctggagatcacaggtggcggtggctcgggcggtggtgggtcgggtggcggcggatctgaggtgaaactgcaggagtcaggacctggcctggtggcgccctcacagagcctgtccgtcacatgcactgtctcaggggtctcattacccgactatggtgtaagctggattcgccagcctccacgaaagggtctggagtggctgggagtaatatggggtagtgaaaccacatactataattcagctctcaaatccagactgaccatcatcaaggacaactccaagagccaagttttcttaaaaatgaacagtctgcaaactgatgacacagccatttactactgtgccaaacattattactacggtggtagctatgctatggactactggggccaaggaacctcagtcaccgtctcctca

SEQ ID NO: 3 - protein, 25 aa, Artificial Sequence
  CD8α跨膜结构域
IYIWAPLAGTCGVLLLSLVITLYCK

SEQ ID NO: 4 - DNA, 75 bp, Artificial Sequence
  CD8α跨膜结构域
atctacatctgggcgcccttggccgggacttgtggggtccttctcctgtcactggttatcaccctttactgcaaa

SEQ ID NO: 5 - protein, 27 aa, Artificial Sequence
  CD28跨膜结构域
FWVLVVVGGVLACYSLLVTVAFIIFWV

SEQ ID NO: 6 - DNA, 81 bp, Artificial Sequence
  CD28跨膜结构域
ttttgggtcctcgtcgtagttggaggggtacttgcctgttatagcctcctggttaccgtagcatttattatattctgggtg

SEQ ID NO: 7 - protein, 41 aa, Artificial Sequence
  CD28胞内区
RSKRSRLLHSDYMNMTPRRPGPTRKHYQPYAPPRDFAAYRS

SEQ ID NO: 8 - DNA, 123 bp, Artificial Sequence
  CD28胞内区
aggagtaagaggagcaggctcctgcacagtgactacatgaacatgactccccgccgccccgggcccacccgcaagcattaccagccctatgccccaccacgcgacttcgcagcctatcgctcc

SEQ ID NO: 9 - protein, 40 aa, Artificial Sequence
  4-1BB胞内区
RGRKKLLYIFKQPFMRPVQTTQEEDGCSCRFPEEEEGGCE

SEQ ID NO: 10 - DNA, 120 bp, Artificial Sequence
  4-1BB胞内区
cggggcagaaagaaactcctgtatatattcaaacaaccatttatgagaccagtacaaactactcaagaggaagatggctgtagctgccgatttccagaagaagaagaaggaggatgtgaa

SEQ ID NO: 11 - protein, 113 aa, Artificial Sequence
  CD3ζ胞内区
LRVKFSRSADAPAYQQGQNQLYNELNLGRREEYDVLDKRRGRDPEMGGKPRRKNPQEGLYNELQKDKMAEAYSEIGMKGERRRGKGHDGLYQGLSTATKDTYDALHMQALPPR

SEQ ID NO: 12 - DNA, 339 bp, Artificial Sequence
  CD3ζ胞内区
ctgagagtgaagttcagcaggagcgcagacgcccccgcgtaccagcagggccagaaccagctctataacgagctcaatctaggacgaagagaggagtacgatgttttggacaagagacgtggccgggaccctgagatggggggaaagccgagaaggaagaaccctcaggaaggcctgtacaatgaactgcagaaagataagatggcggaggcctacagtgagattgggatgaaaggcgagcgccggaggggcaaggggcacgatggcctttaccagggtctcagtacagccaccaaggacacctacgacgcccttcacatgcaggccctgccccctcgc

SEQ ID NO: 13 - protein, 114 aa, Artificial Sequence
  CD3ζ胞内区
LRVKFSRSADAPAYQQGQNQLFNELNLGRREEFDVLDKRRGRDPEMGGKPQRRKNPQEGLYNELQKDKMAEAYSEIGMKGERRRGKGHDGLFQGLSTATKDTFDALHMQALPPR

SEQ ID NO: 14 - DNA, 342 bp, Artificial Sequence
  CD3ζ胞内区
ctgagagtgaagttcagcaggagcgcagacgcccccgcgtaccagcagggccagaaccagctctttaacgagctcaatctaggacgaagagaggagttcgatgttttggacaagagacgtggccgggaccctgagatggggggaaagccgcagagaaggaagaaccctcaggaaggcctgtacaatgaactgcagaaagataagatggcggaggcctacagtgagattgggatgaaaggcgagcgccggaggggcaaggggcacgatggccttttccagggtctcagtacagccaccaaggacacctttgacgcccttcacatgcaggccctgccccctcgc

SEQ ID NO: 15 - protein, 20 aa, Artificial Sequence
  B2M信号肽
MSRSVALAVLALLSLSGLEA

SEQ ID NO: 16 - DNA, 60 bp, Artificial Sequence
  B2M信号肽
atgtcccgctctgttgctttggctgtgctggcccttttgtcccttagcggactggaggcc

SEQ ID NO: 17 - protein, 21 aa, Artificial Sequence
  CD8α信号肽
MALPVTALLLPLALLLHAARP

SEQ ID NO: 18 - DNA, 63 bp, Artificial Sequence
  CD8α信号肽
atggccttaccagtgaccgccttgctcctgccgctggccttgctgctccacgccgccaggccg

SEQ ID NO: 19 - protein, 45 aa, Artificial Sequence
  CD8α铰链区
TTTPAPRPPTPAPTIASQPLSLRPEACRPAAGGAVHTRGLDFACD

SEQ ID NO: 20 - DNA, 135 bp, Artificial Sequence
  CD8α铰链区
accacgacgccagcgccgcgaccaccaacaccggcgcccaccatcgcgtcgcagcccctgtccctgcgcccagaggcgtgccggccagcggcggggggcgcagtgcacacgagggggctggacttcgcctgtgat

SEQ ID NO: 21 - protein, 39 aa, Artificial Sequence
  CD28铰链区
IEVMYPPPYLDNEKSNGTIIHVKGKHLCPSPLFPGPSKP

SEQ ID NO: 22 - DNA, 117 bp, Artificial Sequence
  CD28铰链区
attgaagttatgtatcctcctccttacctagacaatgagaagagcaatggaaccattatccatgtgaaagggaaacacctttgtccaagtcccctatttcccggaccttctaagccc

SEQ ID NO: 23 - protein, 12 aa, Artificial Sequence
  IgG4铰链区
ESKYGPPCPPCP

SEQ ID NO: 24 - DNA, 36 bp, Artificial Sequence
  IgG4铰链区
gaaagcaaatacgggccgccgtgtccaccctgtccg

SEQ ID NO: 25 - protein, 238 aa, Artificial Sequence
  CD19 scFv-2
DIQMTQSPASLSTSLGETVTIQCQASEDIYSGLAWYQQKPGKSPQLLIYGASDLQDGVPSRFSGSGSGTQYSLKITSMQTEDEGVYFCQQGLTYPRTFGGGTKLELKGGGGSGGGGSGGGGSEVQLQQSGAELVRPGTSVKLSCKVSGDTITFYYMHFVKQRPGQGLEWIGRIDPEDESTKYSEKFKNKATLTADTSSNTAYLKLSSLTSEDTATYFCIYGGYYFDYWGQGVMVTVSS

SEQ ID NO: 26 - DNA, 714 bp, Artificial Sequence
  CD19 scFv-2
gacatccagatgacccagagccctgccagcctgtctaccagcctgggcgagacagtgaccatccagtgtcaggccagcgaggacatctactctggcctggcttggtatcagcagaagcccggcaagagccctcagctgctgatctacggcgccagcgacctgcaggacggcgtgcctagcagattcagcggcagcggctccggaacccagtacagcctgaagatcaccagcatgcagaccgaggacgagggcgtgtacttctgccagcaaggcctgacctaccctagaaccttcggaggaggcaccaagctggaactgaagggcggaggcggaagtggaggcggaggatctggcggcggaggctctgaagtgcagctgcagcagtctggcgctgaactggtccggcctggcactagcgtgaagctgtcctgcaaggtgtccggcgacaccatcaccttctactacatgcacttcgtgaagcagaggccaggacagggcctggaatggatcggcagaatcgaccctgaggacgagagcaccaagtacagcgagaagttcaagaacaaggccaccctgaccgccgacaccagcagcaacaccgcctacctgaagctgtctagcctgacctccgaggacaccgccacctacttttgcatctacggcggctactacttcgactactggggccagggcgtgatggtcaccgtgtccagc

SEQ ID NO: 27 - protein, 37 aa, Artificial Sequence
  ICAM3胞内区
REHQRSGSYHVREESTYLPLTSMQPTEAMGEEPSRAE

SEQ ID NO: 28 - DNA, 111 bp, Artificial Sequence
  ICAM3胞内区
cgcgaacaccagagatcagggtcttaccacgtaagagaagaaagtacctaccttcctttgacaagtatgcagccaacggaggctatgggtgaggaaccttccagagcggaa

SEQ ID NO: 29 - protein, 50 aa, Artificial Sequence
  CD155胞内区
SKCSREVLWHCHLCPSSTEHASASANGHVSYSAVSRENSSSQDPQTEGTR

SEQ ID NO: 30 - DNA, 150 bp, Artificial Sequence
  CD155胞内区
tccaaatgttcccgtgaggtcctttggcactgtcatctgtgtccctcgagtacagagcatgccagcgcctcagctaatgggcatgtctcctattcagctgtgagcagagagaacagctcttcccaggatccacagacagagggcacaagg

SEQ ID NO: 31 - protein, 118 aa, Artificial Sequence
  2B4胞内区
RKRKEKQSETSPKEFLTIYEDVKDLKTRRNHEQEQTFPGGGSTIYSMIQSQSSAPTSQEPAYTLYSLIQPSRKSGSRKRNHSPSFNSTIYEVIGKSQPKAQNPARLSRKELENFDVYS

SEQ ID NO: 32 - DNA, 354 bp, Artificial Sequence
  2B4胞内区
agaaagaggaaggagaagcagtcagagaccagtcccaaggaatttttgacaatttacgaagatgtcaaggatctgaaaaccaggagaaatcacgagcaggagcagacttttcctggaggggggagcaccatctactctatgatccagtcccagtcttctgctcccacgtcacaagaacctgcatatacattatattcattaattcagccttccaggaagtctggatccaggaagaggaaccacagcccttccttcaatagcactatctatgaagtgattggaaagagtcaacctaaagcccagaaccctgctcgattgagccgcaaagagctggagaactttgatgtttattcc

SEQ ID NO: 33 - protein, 11 aa, Artificial Sequence
  CD19 scFv-1 CDR-L1
RASQDISKYLN

SEQ ID NO: 34 - protein, 7 aa, Artificial Sequence
  CD19 scFv-1 CDR-L2
HTSRLHS

SEQ ID NO: 35 - protein, 9 aa, Artificial Sequence
  CD19 scFv-1 CDR-L3
QQGNTLPYT

SEQ ID NO: 36 - protein, 7 aa, Artificial Sequence
  CD19 scFv-1 CDR-H1
GVSLPDY

SEQ ID NO: 37 - protein, 5 aa, Artificial Sequence
  CD19 scFv-1 CDR-H2
WGSET

SEQ ID NO: 38 - protein, 12 aa, Artificial Sequence
  CD19 scFv-1 CDR-H3
HYYYGGSYAMDY

SEQ ID NO: 39 - protein, 11 aa, Artificial Sequence
  CD19 scFv-2 CDR-L1
QASEDIYSGLA

SEQ ID NO: 40 - protein, 7 aa, Artificial Sequence
  CD19 scFv-2 CDR-L2
GASDLQD

SEQ ID NO: 41 - protein, 9 aa, Artificial Sequence
  CD19 scFv-2 CDR-L3
QQGLTYPRT

SEQ ID NO: 42 - protein, 7 aa, Artificial Sequence
  CD19 scFv-2 CDR-H1
GDTITFY

SEQ ID NO: 43 - protein, 6 aa, Artificial Sequence
  CD19 scFv-2 CDR-H2
DPEDES

SEQ ID NO: 44 - protein, 7 aa, Artificial Sequence
  CD19 scFv-2 CDR-H3
GGYYFDY